European Patent Application EP 4 295 860 A1, published December 27, 2023. Title: Engineered human T cells comprising a switchable chimeric antigen cell surface receptor and methods for generating them. Applicant: AvenCell Therapeutics Inc. The sequence listing filed with the application follows.

SEQUENCE LISTING (46 sequences)

SEQ ID NO: 1 - RNA, 100 nt, Artificial Sequence
  sgRNA
  misc_feature: contains 2'-O-Me and PS modifications; see specification as filed for detailed description of substitutions
cucucagcugguacacggcaguuuuagagcuagaaauagcaaguuaaaauaaggcuaguccguuaucaacuugaaaaaguggcaccgagucggugcuuuu

SEQ ID NO: 2 - RNA, 100 nt, Artificial Sequence
  sgRNA
  misc_feature: contains 2'-O-Me and PS modifications; see specification as filed for detailed description of substitutions
acagcgacgccgcgagccagguuuuagagcuagaaauagcaaguuaaaauaaggcuaguccguuaucaacuugaaaaaguggcaccgagucggugcuuuu

SEQ ID NO: 3 - RNA, 100 nt, Artificial Sequence
  sgRNA
  misc_feature: contains 2'-O-Me and PS modifications; see specification as filed for detailed description of substitutions
cccccggacgguucaagcaaguuuuagagcuagaaauagcaaguuaaaauaaggcuaguccguuaucaacuugaaaaaguggcaccgagucggugcuuuu

SEQ ID NO: 4 - protein, 5 aa, Artificial Sequence
  linker
GGGGS

SEQ ID NO: 5 - protein, 25 aa, Artificial Sequence
  linker
GGGGSGGGGSGGGGSGGGGSGGGGS

SEQ ID NO: 6 - protein, 25 aa, Artificial Sequence
  linker
GGGGSGGGGSGASAAGGGGSGGGGS

SEQ ID NO: 7 - protein, 33 aa, Saccharomyces cerevisiae
RMKQLEPKVEELLPKNYHLENEVARLKKLVGER

SEQ ID NO: 8 - protein, 14 aa, Saccharomyces cerevisiae
NYHLENEVARLKKL

SEQ ID NO: 9 - protein, 51 aa, Homo sapiens
MDPDLEIRAAFLRQRNTALRTEVAELEQEVQRLENEVSQYETRYGPLGGGK

SEQ ID NO: 10 - protein, 51 aa, Homo sapiens
MDPDLEIEAAFLERENTALETRVAELRQRVQRLRNRVSQYRTRYGPLGGGK

SEQ ID NO: 11 - protein, 10 aa, Homo sapiens
KPLPEVTDEY

SEQ ID NO: 12 - protein, 20 aa, Homo sapiens
  misc_feature (16)..(16): Xaa can be any naturally occurring amino acid
LEKEALKKIIEDQQEXLNKW

SEQ ID NO: 13 - protein, 20 aa, Homo sapiens
LEKEALKKIIEDQQEALNKW

SEQ ID NO: 14 - protein, 113 aa, Artificial Sequence
  Humanized scFv VL chain
  MISC_FEATURE (24)..(24): Xaa can be any naturally occurring amino acid
  MISC_FEATURE (35)..(35): Xaa can be any naturally occurring amino acid
  MISC_FEATURE (61)..(61): Xaa can be any naturally occurring amino acid
  MISC_FEATURE (101)..(101): Xaa can be any naturally occurring amino acid
DIVMTQSPDSLAVSLGERATINCXSSQSLLNSRTXKNYLAWYQQKPGQPPKLLIYWASTRXSGVPDRFSGSGSGTDFTLTISSLQAEDVAVYYCKQSYNLXTFGGGTKVEILK

SEQ ID NO: 15 - protein, 120 aa, Artificial Sequence
  Humanized scFv VH chain
QVQLVQSGAEVKKPGASVKVSCKASGYTFTHYYIYWVRQAPGQGLEWMGGVNPSNGGTHFNEKFKSRVTMTRDTSISTAYMELSRLRSDDTAVYYCARSEYDYGLGFAYWGQGTLVTVSS

SEQ ID NO: 16 - protein, 112 aa, Artificial Sequence
  Humanized scFv VL chain
DIVMTQSPDSLAVSLGERATINCKSSQSLLNSRTPKNYLAWYQQKPGQPPKLLIYWASTRKSGVPDRFSGSGSGTDFTLTISSLQAEDVAVYYCKQSYNLLTFGGGTKVEIK

SEQ ID NO: 17 - protein, 118 aa, Artificial Sequence
  Humanized scFv VH chain
EVQLVESGGGLVQPGGSLRLSCAASGFTFSDFWMNWVRQAPGKGLEWVGQIRNKPNNYETYYSDSLKGRFTISRDDSKSITYLQMNSLRAEDTAVYYCTLGNSWFAYWGQGTLVTVSS

SEQ ID NO: 18 - protein, 112 aa, Artificial Sequence
  Humanized scFv VL chain
DIVMTQSPDSLAVSLGERATINCRSSQSLLDSRTKKNYLAWYQQKPGQPPKLLIYWASTRESGVPDRFSGSGSGTDFTLTISSLQAEDVAVYYCKQSYNLPTFGGGTKVEIK

SEQ ID NO: 19 - protein, 525 aa, Artificial Sequence
  targeting module
EVQLQQSGPELVKPGASVKMSCKASGYTFTDYYMKWVKQSHGKSLEWIGDIIPSNGATFYNQKFKGKATLTVDRSSSTAYMHLNSLTSEDSAVYYCTRSHLLRASWFAYWGQGTLVTVSAASGGGGSGGGGSGGGGSDFVMTQSPSSLTVTAGEKVTMSCKSSQSLLNSGNQKNYLTWYLQKPGQPPKLLIYWASTRESGVPDRFTGSGSGTDFTLTISSVQAEDLAVYYCQNDYSYPYTFGGGTKLEIKAAARGQVQLVQSGAEVKKPGASVKVSCKASGYTFTHYYIYWVRQAPGQGLEWMGGVNPSNGGTHFNEKFKSRVTMTRDTSISTAYMELSRLRSDDTAVYYCARSEYDYGLGFAYWGQGTLVTVSSGGGGSGGGGSGGGGSDIVMTQSPDSLAVSLGERATINCKSSQSLLNSRTPKNYLAWYQQKPGQPPKLLIYWASTRKSGVPDRFSGSGSGTDFTLTISSLQAEDVAVYYCKQSYNLLTFGGGTKVEIKGPEQKLISEEDLNSAVDHHHHHH

SEQ ID NO: 20 - protein, 516 aa, Artificial Sequence
  targeting module
GQVQLVQSGAEVKKPGASVKVSCKASGYTFTDYYMHWVRQAPGQGLEWMGDIIPSNGATFYAQKFQGRVTMTRDTSTSTVYMELSSLRSEDTAVYYCTRSHLLRASWFAYWGQGTLVTVSSASGGGGSGGGGSGGGGSDIVMTQSPDSLAVSLGERATINCKSSQSLLNSGNQKNYLAWYQQKPGQPPKLLIYWASTRESGVPDRFSGSGSGTDFTLTISSLQAEDVAVYYCQNDYSYPYTFGGGTKLEIKAAARGQVQLVQSGAEVKKPGASVKVSCKASGYTFTHYYIYWVRQAPGQGLEWMGGVNPSNGGTHFNEKFKSRVTMTRDTSISTAYMELSRLRSDDTAVYYCARSEYDYGLGFAYWGQGTLVTVSSGGGGSGGGGSGGGGSDIVMTQSPDSLAVSLGERATINCKSSQSLLNSRTPKNYLAWYQQKPGQPPKLLIYWASTRKSGVPDRFSGSGSGTDFTLTISSLQAEDVAVYYCKQSYNLLTFGGGTKVEIKGGGGSHHHHHHHH

SEQ ID NO: 21 - protein, 526 aa, Artificial Sequence
  targeting module
GQVQLVQSGAEVKKPGSSVKVSCKASGYTFTDYYIHWVRQAPGQGLEWMGDIIPSNGATFYNQRFKGRVTITADESTSTAYMELSSLRSEDTAVYYCTRSHLLRASWFAYWGQGTLVTVSSASGGGGSGGGGSGGGGSDIVMTQTPLSLSVTPGQPASISCRSSQSLLNSGNQKNYLTWYLQKPGQSPQLLIYWASTRFIGVPDRFSGSGSGTDFTLKISRVEAEDVGVYYCQNDYSYPYTFGQGTKLEIKAAARGDIVMTQSPDSLAVSLGERATINCKSSQSLLNSRTPKNYLAWYQQKPGQPPKLLIYWASTRKSGVPDRFSGSGSGTDFTLTISSLQAEDVAVYYCKQSYNLLTFGGGTKVEIKGGGGSGGGGSGASAAGGGGSGGGGSQVQLVQSGAEVKKPGASVKVSCKASGYTFTHYYIYWVRQAPGQGLEWMGGVNPSNGGTHFNEKFKSRVTMTRDTSISTAYMELSRLRSDDTAVYYCARSEYDYGLGFAYWGQGTLVTVSSGGGGSHHHHHHHH

SEQ ID NO: 22 - protein, 526 aa, Artificial Sequence
  targeting module
GQVQLVQSGAEVKKPGASVKMSCKASGYTFTDYYMKWVKQAPGQGLEWIGDIIPSNGATFYNQKFQGRATLTVDTSTSTAYMELSSLRSEDTAVYYCTRSHLLRASWFAYWGQGTLVTVSSASGGGGSGGGGSGGGGSDIVMTQSPDSLAVSLGERATINCKSSQSLLNSGNQKNYLTWYLQKPGQPPKLLIYWASTRESGVPDRFSGSGSGTDFTLTISSVQAEDVAVYYCQNDYSYPYTFGGGTKLEIKAAARGDIVMTQSPDSLAVSLGERVTMNCKSSQSLLNSRTPKNYLAWYQQKPGQSPKLLIYWASTRKSGVPDRFSGSGSGTDFTLTISSVQAEDVAVYYCKQSYNLLTFGGGTKLEIKGGGGSGGGGSGASAAGGGGSGGGGSQVQLVESGAEVVKPGASVKLSCKASGYAFTHYYIYWIKQAPGQGLEWIGGVNPSNGGTHFNEKFKSRATLTVDTSISTAYMELSRLRSDDTAVYYCTRSEYDYGLGFAYWGQGTLVTVSSGGGGSHHHHHHHH

SEQ ID NO: 23 - protein, 515 aa, Artificial Sequence
  targeting module
EVQLQQSGPELVKPGASVKMSCKASGYTFTDYYMKWVKQSHGKSLEWIGDIIPSNGATFYNQKFKGKATLTVDRSSSTAYMHLNSLTSEDSAVYYCTRSHLLRASWFAYWGQGTLVTVSAASGGGGSGGGGSGGGGSDFVMTQSPSSLTVTAGEKVTMSCKSSQSLLNSGNQKNYLTWYLQKPGQPPKLLIYWASTRESGVPDRFTGSGSGTDFTLTISSVQAEDLAVYYCQNDYSYPYTFGGGTKLEIKAAARGQVQLVQSGAEVKKPGASVKVSCKASGYTFTHYYIYWVRQAPGQGLEWMGGVNPSNGGTHFNEKFKSRVTMTRDTSISTAYMELSRLRSDDTAVYYCARSEYDYGLGFAYWGQGTLVTVSSGGGGSGGGGSGGGGSDIVMTQSPDSLAVSLGERATINCKSSQSLLNSRTPKNYLAWYQQKPGQPPKLLIYWASTRKSGVPDRFSGSGSGTDFTLTISSLQAEDVAVYYCKQSYNLLTFGGGTKVEIKGGGGSHHHHHHHH

SEQ ID NO: 24 - protein, 525 aa, Artificial Sequence
  targeting module
EVQLQQSGPELVKPGASVKMSCKASGYTFTDYYMKWVKQSHGKSLEWIGDIIPSNGATFYNQKFKGKATLTVDRSSSTAYMHLNSLTSEDSAVYYCTRSHLLRASWFAYWGQGTLVTVSAASGGGGSGGGGSGGGGSDFVMTQSPSSLTVTAGEKVTMSCKSSQSLLNSGNQKNYLTWYLQKPGQPPKLLIYWASTRESGVPDRFTGSGSGTDFTLTISSVQAEDLAVYYCQNDYSYPYTFGGGTKLEIKAAARGDIVMTQSPDSLAVSLGERATINCKSSQSLLNSRTPKNYLAWYQQKPGQPPKLLIYWASTRKSGVPDRFSGSGSGTDFTLTISSLQAEDVAVYYCKQSYNLLTFGGGTKVEIKGGGGSGGGGSGASAAGGGGSGGGGSQVQLVQSGAEVKKPGASVKVSCKASGYTFTHYYIYWVRQAPGQGLEWMGGVNPSNGGTHFNEKFKSRVTMTRDTSISTAYMELSRLRSDDTAVYYCARSEYDYGLGFAYWGQGTLVTVSSGGGGSHHHHHHHH

SEQ ID NO: 25 - protein, 525 aa, Artificial Sequence
  targeting module
EVQLQQSGPELVKPGASVKMSCKASGYTFTDYYMKWVKQSHGKSLEWIGDIIPSNGATFYNQKFKGKATLTVDRSSSTAYMHLNSLTSEDSAVYYCTRSHLLRASWFAYWGQGTLVTVSAASGGGGSGGGGSGGGGSDFVMTQSPSSLTVTAGEKVTMSCKSSQSLLNSGNQKNYLTWYLQKPGQPPKLLIYWASTRESGVPDRFTGSGSGTDFTLTISSVQAEDLAVYYCQNDYSYPYTFGGGTKLEIKAAARGDIVMTQSPDSLAVSLGERVTMNCKSSQSLLNSRTPKNYLAWYQQKPGQSPKLLIYWASTRKSGVPDRFSGSGSGTDFTLTISSVQAEDVAVYYCKQSYNLLTFGGGTKLEIKGGGGSGGGGSGASAAGGGGSGGGGSQVQLVESGAEVVKPGASVKLSCKASGYAFTHYYIYWIKQAPGQGLEWIGGVNPSNGGTHFNEKFKSRATLTVDTSISTAYMELSRLRSDDTAVYYCTRSEYDYGLGFAYWGQGTLVTVSSGGGGSHHHHHHHH

SEQ ID NO: 26 - protein, 516 aa, Artificial Sequence
  targeting module
GQVQLVQSGAEVKKPGSSVKVSCKASGYTFTDYYIHWVRQAPGQGLEWMGDIIPSNGATFYNQRFKGRVTITADESTSTAYMELSSLRSEDTAVYYCTRSHLLRASWFAYWGQGTLVTVSSASGGGGSGGGGSGGGGSDIVMTQTPLSLSVTPGQPASISCRSSQSLLNSGNQKNYLTWYLQKPGQSPQLLIYWASTRFIGVPDRFSGSGSGTDFTLKISRVEAEDVGVYYCQNDYSYPYTFGQGTKLEIKAAARGQVQLVQSGAEVKKPGASVKVSCKASGYTFTHYYIYWVRQAPGQGLEWMGGVNPSNGGTHFNEKFKSRVTMTRDTSISTAYMELSRLRSDDTAVYYCARSEYDYGLGFAYWGQGTLVTVSSGGGGSGGGGSGGGGSDIVMTQSPDSLAVSLGERATINCKSSQSLLNSRTPKNYLAWYQQKPGQPPKLLIYWASTRKSGVPDRFSGSGSGTDFTLTISSLQAEDVAVYYCKQSYNLLTFGGGTKVEIKGGGGSHHHHHHHH

SEQ ID NO: 27 - protein, 516 aa, Artificial Sequence
  targeting module
GQVQLVQSGAEVKKPGASVKMSCKASGYTFTDYYMKWVKQAPGQGLEWIGDIIPSNGATFYNQKFQGRATLTVDTSTSTAYMELSSLRSEDTAVYYCTRSHLLRASWFAYWGQGTLVTVSSASGGGGSGGGGSGGGGSDIVMTQSPDSLAVSLGERATINCKSSQSLLNSGNQKNYLTWYLQKPGQPPKLLIYWASTRESGVPDRFSGSGSGTDFTLTISSVQAEDVAVYYCQNDYSYPYTFGGGTKLEIKAAARGQVQLVQSGAEVKKPGASVKVSCKASGYTFTHYYIYWVRQAPGQGLEWMGGVNPSNGGTHFNEKFKSRVTMTRDTSISTAYMELSRLRSDDTAVYYCARSEYDYGLGFAYWGQGTLVTVSSGGGGSGGGGSGGGGSDIVMTQSPDSLAVSLGERATINCKSSQSLLNSRTPKNYLAWYQQKPGQPPKLLIYWASTRKSGVPDRFSGSGSGTDFTLTISSLQAEDVAVYYCKQSYNLLTFGGGTKVEIKGGGGSHHHHHHHH

SEQ ID NO: 28 - protein, 526 aa, Artificial Sequence
  targeting module
GQVQLVQSGAEVKKPGASVKMSCKASGYTFTDYYMKWVKQAPGQGLEWIGDIIPSNGATFYNQKFQGRATLTVDTSTSTAYMELSSLRSEDTAVYYCTRSHLLRASWFAYWGQGTLVTVSSASGGGGSGGGGSGGGGSDIVMTQSPDSLAVSLGERATINCKSSQSLLNSGNQKNYLTWYLQKPGQPPKLLIYWASTRESGVPDRFSGSGSGTDFTLTISSVQAEDVAVYYCQNDYSYPYTFGGGTKLEIKAAARGDIVMTQSPDSLAVSLGERATINCKSSQSLLNSRTPKNYLAWYQQKPGQPPKLLIYWASTRKSGVPDRFSGSGSGTDFTLTISSLQAEDVAVYYCKQSYNLLTFGGGTKVEIKGGGGSGGGGSGASAAGGGGSGGGGSQVQLVQSGAEVKKPGASVKVSCKASGYTFTHYYIYWVRQAPGQGLEWMGGVNPSNGGTHFNEKFKSRVTMTRDTSISTAYMELSRLRSDDTAVYYCARSEYDYGLGFAYWGQGTLVTVSSGGGGSHHHHHHHH

SEQ ID NO: 29 - protein, 526 aa, Artificial Sequence
  targeting module
GQVQLVQSGAEVKKPGASVKMSCKASGYTFTDYYMKWVKQAPGQGLEWIGDIIPSNGATFYNQKFKGRATLTVDKSTSTAYMELSSLRSEDTAVYYCTRSHLLRASWFAYWGQGTLVTVSSASGGGGSGGGGSGGGGSDFVMTQSPDSLAVSLGERATMNCKSSQSLLNSGNQKNYLTWYLQKPGQPPKLLIYWASTRESGVPDRFSGSGSGTDFTLTISSVQAEDVAVYYCQNDYSYPYTFGGGTKLEIKAAARGQVQLVQSGAEVKKPGASVKVSCKASGYTFTHYYIYWVRQAPGQGLEWMGGVNPSNGGTHFNEKFKSRVTMTRDTSISTAYMELSRLRSDDTAVYYCARSEYDYGLGFAYWGQGTLVTVSSGGGGSGGGGSGASAAGGGGSGGGGSDIVMTQSPDSLAVSLGERATINCKSSQSLLNSRTPKNYLAWYQQKPGQPPKLLIYWASTRKSGVPDRFSGSGSGTDFTLTISSLQAEDVAVYYCKQSYNLLTFGGGTKVEIKGGGGSHHHHHHHH

SEQ ID NO: 30 - protein, 526 aa, Artificial Sequence
  targeting module
GQVQLVQSGAEVKKPGASVKMSCKASGYTFTDYYMKWVKQAPGQGLEWIGDIIPSNGATFYNQKFKGRATLTVDKSTSTAYMELSSLRSEDTAVYYCTRSHLLRASWFAYWGQGTLVTVSSASGGGGSGGGGSGGGGSDFVMTQSPDSLAVSLGERATMNCKSSQSLLNSGNQKNYLTWYLQKPGQPPKLLIYWASTRESGVPDRFSGSGSGTDFTLTISSVQAEDVAVYYCQNDYSYPYTFGGGTKLEIKAAARGDIVMTQSPDSLAVSLGERATINCKSSQSLLNSRTPKNYLAWYQQKPGQPPKLLIYWASTRKSGVPDRFSGSGSGTDFTLTISSLQAEDVAVYYCKQSYNLLTFGGGTKVEIKGGGGSGGGGSGASAAGGGGSGGGGSQVQLVQSGAEVKKPGASVKVSCKASGYTFTHYYIYWVRQAPGQGLEWMGGVNPSNGGTHFNEKFKSRVTMTRDTSISTAYMELSRLRSDDTAVYYCARSEYDYGLGFAYWGQGTLVTVSSGGGGSHHHHHHHH

SEQ ID NO: 31 - protein, 525 aa, Artificial Sequence
  targeting module
EVQLVQSGAEVKKPGASVKMSCKASGYTFTDYYMKWVKQAPGQGLEWIGDIIPSNGATFYNQKFKGRATLTVDRSTSTAYMELSSLRSEDTAVYYCTRSHLLRASWFAYWGQGTLVTVSSASGGGGSGGGGSGGGGSDFVMTQSPDSLAVSLGERATINCESSQSLLNTGNQKNYLTWYLQKPGQPPKLLIYWASTRESGVPDRFSGSGSGTDFTLTISSVQAEDVAVYYCQNDYSYPYTFGGGTKLEIKAAARGDIVMTQSPDSLAVSLGERATINCKSSQSLLNSRTPKNYLAWYQQKPGQPPKLLIYWASTRKSGVPDRFSGSGSGTDFTLTISSLQAEDVAVYYCKQSYNLLTFGGGTKVEIKGGGGSGGGGSGASAAGGGGSGGGGSQVQLVQSGAEVKKPGASVKVSCKASGYTFTHYYIYWVRQAPGQGLEWMGGVNPSNGGTHFNEKFKSRVTMTRDTSISTAYMELSRLRSDDTAVYYCARSEYDYGLGFAYWGQGTLVTVSSGGGGSHHHHHHHH

SEQ ID NO: 32 - protein, 525 aa, Artificial Sequence
  targeting module
EVQLVQSGAEVKKPGASVKMSCKASGYTFTDYYMKWVKQAPGQGLEWIGDIIPSNGATFYNQKFKGRATLTVDRSTSTAYMELSSLRSEDTAVYYCTRSHLLRASWFAYWGQGTLVTVSSASGGGGSGGGGSGGGGSDFVMTQSPDSLAVSLGERATINCESSQSLLNTGNQKNYLTWYLQKPGQPPKLLIYWASTRESGVPDRFSGSGSGTDFTLTISSVQAEDVAVYYCQNDYSYPYTFGGGTKLEIKAAARGDIVMTQSPDSLAVSLGERVTMNCKSSQSLLNSRTPKNYLAWYQQKPGQSPKLLIYWASTRKSGVPDRFSGSGSGTDFTLTISSVQAEDVAVYYCKQSYNLLTFGGGTKLEIKGGGGSGGGGSGASAAGGGGSGGGGSQVQLVESGAEVVKPGASVKLSCKASGYAFTHYYIYWIKQAPGQGLEWIGGVNPSNGGTHFNEKFKSRATLTVDTSISTAYMELSRLRSDDTAVYYCTRSEYDYGLGFAYWGQGTLVTVSSGGGGSHHHHHHHH

SEQ ID NO: 33 - protein, 367 aa, Artificial Sequence
  humanized homo sapiens/mus musculus chimera
MRRMQLLLLIALSLALVTNSEFKPLPEVTDEYAAAGPGGGGSKILVKQSPMLVAYDNAVNLSCKYSYNLFSREFRASLHKGLDSAVEVCVVYGNYSQQLQVYSKTGFNCDGKLGNESVTFYLQNLYVNQTDIYFCKIEVMAPPPALDNEKSNGTIIHVKGKHLCPSPLFPGPSKPFWVLVVVGGVLACYSLLVTVAFIIFWVRSKRSRGGHSDYMNMTPRRPGPTRKHYQPYAPPRDFAAYRSGGGGSGGGASGGGGSFSRSADAPAYQQGQNQLYNELNLGRREEYDVLDKRRGRDPEMGGKPRRKNPQEGLYNELQKDKMAEAYSEIGMKGERRRGKGHDGLYQGLSTATKDTYGALHMQALPPR

SEQ ID NO: 34 - protein, 379 aa, Artificial Sequence
  humanized homo sapiens/mus musculus chimera
MRRMQLLLLIALSLALVTNSEFKPLPEVTDEYAAAGPGGGGSKILVKQSPMLVAYDNAVNLSCKYSYNLFSREFRASLHKGLDSAVEVCVVYGNYSQQLQVYSKTGFNCDGKLGNESVTFYLQNLYVNQTDIYFCKIEVMAPPPALDNEKSNGTIIHVKGKHLCPSPLFPGPSKPFWVLVVVGGVLACYSLLVTVAFIIFWVRSKRSRGGGGSKRGRKKLLYIFKQPFMRPVQTTQEEDGCSCRFPEEEEGGCELGGGGSGGGASGGGGSFSRSADAPAYQQGQNQLYNELNLGRREEYDVLDKRRGRDPEMGGKPRRKNPQEGLYNELQKDKMAEAYSEIGMKGERRRGKGHDGLYQGLSTATKDTYGALHMQALPPR

SEQ ID NO: 35 - protein, 375 aa, Artificial Sequence
  humanized homo sapiens/mus musculus chimera
MRRMQLLLLIALSLALVTNSEFEKEALKKIIEDQQESLNKAAAGPGGGGSKILVKQSPMLVAYDNAVNLSCKYSYNLFSREFRASLHKGLDSAVEVCVVYGNYSQQLQVYSKTGFNCDGKLGNESVTFYLQNLYVNQTDIYFCKIEVMAPPPALDNEKSNGTIIHVKGKHLCPSPLFPGPSKPFWVLVVVGGVLACYSLLVTVAFIIFWVRSKRSRGGHSDYMNMTPRRPGPTRKHYQPYAPPRDFAAYRSGGGGSGGGASGGGGSFSRSADAPAYQQGQNQLYNELNLGRREEYDVLDKRRGRDPEMGGKPRRKNPQEGLYNELQKDKMAEAYSEIGMKGERRRGKGHDGLYQGLSTATKDTYGALHMQALPPR

SEQ ID NO: 36 - protein, 387 aa, Artificial Sequence
  humanized homo sapiens/mus musculus chimera
MRRMQLLLLIALSLALVTNSEFEKEALKKIIEDQQESLNKAAAGPGGGGSKILVKQSPMLVAYDNAVNLSCKYSYNLFSREFRASLHKGLDSAVEVCVVYGNYSQQLQVYSKTGFNCDGKLGNESVTFYLQNLYVNQTDIYFCKIEVMAPPPALDNEKSNGTIIHVKGKHLCPSPLFPGPSKPFWVLVVVGGVLACYSLLVTVAFIIFWVRSKRSRGGGGSKRGRKKLLYIFKQPFMRPVQTTQEEDGCSCRFPEEEEGGCELGGGGSGGGASGGGGSFSRSADAPAYQQGQNQLYNELNLGRREEYDVLDKRRGRDPEMGGKPRRKNPQEGLYNELQKDKMAEAYSEIGMKGERRRGKGHDGLYQGLSTATKDTYGALHMQALPPR

SEQ ID NO: 37 - DNA, 1101 bp, Artificial Sequence
  humanized homo sapiens/mus musculus chimera
atgcgccgcatgcagctgctgcttctgatcgctctgagcctggctcttgtgaccaactctgaattcaaacccctacctgaagtgactgatgagtatgctgccgctgggcccggaggaggcggcagcaagatcctggtcaaacagtcccctatgctggtcgcttacgacaacgccgttaatctgagttgcaaatatagttacaacctgtttagccgggaatttcgcgcatctctccacaagggactggattctgcggttgaggtttgtgtggtctatggcaattatagccagcaactgcaagtgtacagcaaaacaggctttaactgcgacgggaaactcgggaacgaatcagtgaccttctatctgcagaacctgtacgttaaccaaacagatatttacttctgcaagatagaggtgatggctccaccgccagcactggataacgagaagtccaatggaaccatcattcacgtcaaggggaagcatctgtgtccttccccgttgttccctgggccgagcaaacccttttgggtgcttgtggtagttggcggggtattggcctgctattcccttctcgtaactgtggccttcatcatcttctgggtcagatctaagaggtctaggggcgggcatagcgactacatgaacatgacacccaggcggcctggccccactcgcaaacactaccagccatacgcaccaccaagagactttgccgcatatcggagtggtggcggcgggtcaggaggtggagctagcggtggaggaggttccttctctaggtcagctgatgctcccgcctatcagcaaggtcagaaccagctctacaatgagctgaatctgggacgtcgggaggagtacgacgtgctggataaacgaagaggacgcgatcccgagatgggtgggaagcctaggcgcaagaatccccaggaaggcctctacaatgaactgcagaaagacaagatggccgaagcctacagcgagattggcatgaaaggggagcgacggagaggaaagggacatgacgggttgtatcagggtctttccactgcgacaaaggatacctatggggctctgcacatgcaagcactgccacctaga

SEQ ID NO: 38 - DNA, 1137 bp, Artificial Sequence
  humanized homo sapiens/mus musculus chimera
atgcgccgcatgcagctgctgcttctgatcgctctgagcctggctcttgtgaccaactctgaattcaaacccctacctgaagtgactgatgagtatgctgccgctgggcccggaggaggcggcagcaagatcctggtcaaacagtcccctatgctggtcgcttacgacaacgccgttaatctgagttgcaaatatagttacaacctgtttagccgggaatttcgcgcatctctccacaagggactggattctgcggttgaggtttgtgtggtctatggcaattatagccagcaactgcaagtgtacagcaaaacaggctttaactgcgacgggaaactcgggaacgaatcagtgaccttctatctgcagaacctgtacgttaaccaaacagatatttacttctgcaagatagaggtgatggctccaccgccagcactggataacgagaagtccaatggaaccatcattcacgtcaaggggaagcatctgtgtccttccccgttgttccctgggccgagcaaacccttttgggtgcttgtggtagttggcggggtattggcctgctattcccttctcgtaactgtggccttcatcatcttctgggtcagatctaagaggtctaggggcgggggcgggtcaaaacgcggacggaagaaactgctgtacatcttcaagcagcccttcatgcgccccgtgcagacaacacaggaagaggacggttgcagctgccgatttcccgaagaggaggagggaggctgtgaattgggtggcggcgggtcaggaggtggagctagcggtggaggaggttccttctctaggtcagctgatgctcccgcctatcagcaaggtcagaaccagctctacaatgagctgaatctgggacgtcgggaggagtacgacgtgctggataaacgaagaggacgcgatcccgagatgggtgggaagcctaggcgcaagaatccccaggaaggcctctacaatgaactgcagaaagacaagatggccgaagcctacagcgagattggcatgaaaggggagcgacggagaggaaagggacatgacgggttgtatcagggtctttccactgcgacaaaggatacctatggggctctgcacatgcaagcactgccacctaga

SEQ ID NO: 39 - DNA, 1125 bp, Artificial Sequence
  humanized homo sapiens/mus musculus chimera
atgcgccgcatgcagctgctgcttctgatcgctctgagcctggctcttgtgaccaactctgaattcgagaaagaagcactgaagaaaataatagaagaccaacaagaatccctaaacaaagctgccgctgggcccggaggaggcggcagcaagatcctggtcaaacagtcccctatgctggtcgcttacgacaacgccgttaatctgagttgcaaatatagttacaacctgtttagccgggaatttcgcgcatctctccacaagggactggattctgcggttgaggtttgtgtggtctatggcaattatagccagcaactgcaagtgtacagcaaaacaggctttaactgcgacgggaaactcgggaacgaatcagtgaccttctatctgcagaacctgtacgttaaccaaacagatatttacttctgcaagatagaggtgatggctccaccgccagcactggataacgagaagtccaatggaaccatcattcacgtcaaggggaagcatctgtgtccttccccgttgttccctgggccgagcaaacccttttgggtgcttgtggtagttggcggggtattggcctgctattcccttctcgtaactgtggccttcatcatcttctgggtcagatctaagaggtctaggggcgggcatagcgactacatgaacatgacacccaggcggcctggccccactcgcaaacactaccagccatacgcaccaccaagagactttgccgcatatcggagtggtggcggcgggtcaggaggtggagctagcggtggaggaggttccttctctaggtcagctgatgctcccgcctatcagcaaggtcagaaccagctctacaatgagctgaatctgggacgtcgggaggagtacgacgtgctggataaacgaagaggacgcgatcccgagatgggtgggaagcctaggcgcaagaatccccaggaaggcctctacaatgaactgcagaaagacaagatggccgaagcctacagcgagattggcatgaaaggggagcgacggagaggaaagggacatgacgggttgtatcagggtctttccactgcgacaaaggatacctatggggctctgcacatgcaagcactgccacctaga

SEQ ID NO: 40 - DNA, 1161 bp, Artificial Sequence
  humanized homo sapiens/mus musculus chimera
atgcgccgcatgcagctgctgcttctgatcgctctgagcctggctcttgtgaccaactctgaattcgagaaagaagcactgaagaaaataatagaagaccaacaagaatccctaaacaaagctgccgctgggcccggaggaggcggcagcaagatcctggtcaaacagtcccctatgctggtcgcttacgacaacgccgttaatctgagttgcaaatatagttacaacctgtttagccgggaatttcgcgcatctctccacaagggactggattctgcggttgaggtttgtgtggtctatggcaattatagccagcaactgcaagtgtacagcaaaacaggctttaactgcgacgggaaactcgggaacgaatcagtgaccttctatctgcagaacctgtacgttaaccaaacagatatttacttctgcaagatagaggtgatggctccaccgccagcactggataacgagaagtccaatggaaccatcattcacgtcaaggggaagcatctgtgtccttccccgttgttccctgggccgagcaaacccttttgggtgcttgtggtagttggcggggtattggcctgctattcccttctcgtaactgtggccttcatcatcttctgggtcagatctaagaggtctaggggcgggggcgggtcaaaacgcggacggaagaaactgctgtacatcttcaagcagcccttcatgcgccccgtgcagacaacacaggaagaggacggttgcagctgccgatttcccgaagaggaggagggaggctgtgaattgggtggcggcgggtcaggaggtggagctagcggtggaggaggttccttctctaggtcagctgatgctcccgcctatcagcaaggtcagaaccagctctacaatgagctgaatctgggacgtcgggaggagtacgacgtgctggataaacgaagaggacgcgatcccgagatgggtgggaagcctaggcgcaagaatccccaggaaggcctctacaatgaactgcagaaagacaagatggccgaagcctacagcgagattggcatgaaaggggagcgacggagaggaaagggacatgacgggttgtatcagggtctttccactgcgacaaaggatacctatggggctctgcacatgcaagcactgccacctaga

SEQ ID NO: 41 - RNA, 20 nt, Artificial Sequence
  guide sequence
cucucagcugguacacggca

SEQ ID NO: 42 - RNA, 20 nt, Artificial Sequence
  guide sequence
acagcgacgccgcgagccag

SEQ ID NO: 43 - RNA, 20 nt, Artificial Sequence
  guide sequence
cccccggacgguucaagcaa

SEQ ID NO: 44 - RNA, 100 nt, Artificial Sequence; identical to SEQ ID NO: 1
  guide RNA sequence

SEQ ID NO: 45 - RNA, 100 nt, Artificial Sequence; identical to SEQ ID NO: 2
  guide RNA sequence

SEQ ID NO: 46 - RNA, 100 nt, Artificial Sequence; identical to SEQ ID NO: 3
  guide RNA sequence